European Patent Application EP 4 755 901 A1, published June 10, 2026. Title: A novel promoter and method for producing L-isoleucine using thereof. Applicant: CJ CheilJedang Corporation. The sequence listing filed with the application follows.

SEQUENCE LISTING (61 sequences)

SEQ ID NO: 1 - DNA, 396 bp, synthetic construct
  misc_feature 1..396: note = Pn*_NCgl0867
  source 1..396: mol_type = other DNA
gacgtcaaaaggttttagcactataacgttatgacgttttagtgctaaagtgtggcttgtcagattcgtgttggtcgtgcgcccgtatggtgatttgagacagggtttaggagaattagttccatgtcgaatcgcacgtcatcttcaccgaagaattcaaagcaggagctgtgcaactcgtcgtatcctcagggcgctcggtcaaggaagtggccaccgagttgggtatcaaagaaggaacactgagcgcgtgggtaagaacctggagggccgagcatccagacgccggtgtggatgaaccaggcccagtcgaatgggcgaaatacaaggccctgcaggctgagaacgccgcgttgaaacgggaaaacgagttttggggaaaagccagcgccttct

SEQ ID NO: 2 - DNA, 164 bp, synthetic construct
  misc_feature 1..164: note = Pn*_NCgl1062
  source 1..164: mol_type = other DNA
cccccatttggttcgcagccgatgaggagttacgcactatcgactccatcgaaggccaagcaaattggtcaatcaagcgtgaatccggcttccatgagccagttgcccgcctcaaagcttgacccattttcataatcagtgccatgtgggtttacggttgatac

SEQ ID NO: 3 - DNA, 164 bp, synthetic construct
  misc_feature 1..164: note = Pn*_NCgl2412
  source 1..164: mol_type = other DNA
ctaggacactggaacctaaatccagcgcgtctgccaattccgccacaagcgcttaatgcgggttttactatacatggtgtagtcccaaattaactaatccgggtgaccaactgcaccgtaaaaaaaattcgcttatcgtaaatcagcaggtagaataacactct

SEQ ID NO: 4 - DNA, 180 bp, synthetic construct
  misc_feature 1..180: note = Pn*_NCgl1224
  source 1..180: mol_type = other DNA
acagcaattaatctgattgcacctgctgcataaatgtggctagtcaaacaccgtctaattacatgtgtgtggtagaacaataatgtagttgtctgcccaagcgagttaaactcccacgatttacagtggggggcagacatcttttcaccaaaatttttacgaaaggcgagattttctccc

SEQ ID NO: 5 - DNA, 232 bp, synthetic construct
  misc_feature 1..232: note = Pn*_NCgl2581
  source 1..232: mol_type = other DNA
aaatttgtgggaaccgaccgacaagtccgcggcctgatcatggacgtgctgcgcaatgccaccgcacctgtgccactatccgcgattgatgtcgtgtggcctgacgatgcccaacgctcccgggcgctgttttcgctcattgaggacggactcgcggaacaagatgaggcgggttatttccacctgccacgataaaacactgcgcgcctgcaaaaaacagtaggtttaagta

SEQ ID NO: 6 - DNA, 326 bp, synthetic construct
  misc_feature 1..326: note = Pn*_NCgl2658
  source 1..326: mol_type = other DNA
agcacaaatgcttattgccgtagataacaatacggagcggttacaagttgcgaagcaccctttgcaaagtttttagcggtactttacagctcttcaccccccattaatggggtctatgaaagcgcgcagcgtgacaaatctgaccccagcaaagcccccaatactccccgactggcctttattagtctgcacttaccacgtatcatggagggttgatagcagggcaccattagcagtcgcaccccgataggagtcgaatctacaagtggaacccccgctcacatactccacattttttagaacccctttaaggaatcgaactttat

SEQ ID NO: 7 - DNA, 235 bp, synthetic construct
  misc_feature 1..235: note = Pn*_NCgl2046
  source 1..235: mol_type = other DNA
agtacttcgacgcaaagacaaaacttttctcctggcaataaatatgcggatttactatggaaacaagatagaagattggatagcgaaagctatcctcaactcgtggaaagtgtagtgccacaaccacagtattggctagaaaacaatctatagcattgttctacaaagagcttgttggaaataaaacctatgccaaagtaggtgcaattctaggagtgtggtataatggtcaacc

SEQ ID NO: 8 - DNA, 184 bp, synthetic construct
  misc_feature 1..184: note = Pn*_NCgl0780
  source 1..184: mol_type = other DNA
ggggtgtggtggatacacatggttgtgtgttcaccgcaccctctctttttttgtgtttgtgggggtcttgggccccttgtgcacgtggcacctgcgcctgggggcaagcgtcgacaagcacaaactttttgcttaattgaatcctttgcgcaccaatcaatgggggatcaaatatagtagctgc

SEQ ID NO: 9 - DNA, 200 bp, synthetic construct
  misc_feature 1..200: note = Pn*_NCgl1896
  source 1..200: mol_type = other DNA
cgcaaagctcacacccacgagctaaaaattcatatagttaagacaacatttttggctgtaaaagacagccgtaaaaacctcttgctcgtgtcaattgttcttatcggaatgtggcttgggcgattgttatgcaaaagttgttaggttttttgcgtggttgttgggcccccaaatgagggaagaaggtaaccttgaactct

SEQ ID NO: 10 - DNA, 284 bp, synthetic construct
  misc_feature 1..284: note = Pn*_NCgl2356
  source 1..284: mol_type = other DNA
gttttctagataacaaggccagcacagaccaccatatctacgaccccaaaaaccgactccaagctccgcggcgacgaagccgcgctcgcgccaccgaccaagcagccggtccaggtttaaagattttgcttttcgacgctcccctccacctcattcaatgcggcgggaggggatttccttgcatgttaagcctataggaaaaagtgtttgcatatcacccttgtattcgaacacgtgagcgggtagagtgggtggtaacaacacggggaaagggggaagacacc

SEQ ID NO: 11 - DNA, 5802 bp, synthetic construct
  misc_feature 1..5802: note = PDC24 vector
  source 1..5802: mol_type = other DNA
gttcgcttgctgtccataaaaccgcccagtctagctatcgccatgtaagcccactgcaagctacctgctttctctttgcgcttgcgttttcccttgtccagatagcccagtagctgacattcatccggggtcagcaccgtttctgcggactggctttctacgtgttccgcttcctttagcagcccttgcgccctgagtgcttgcggcagcgtgaagctagcttttatcgccattcgccattcaggctgcgcaactgttgggaagggcgatcggtgcgggcctcttcgctattacgccagctggcgaaagggggatgtgctgcaaggcgattaagttgggtaacgccagggttttcccagtcacgacgttgtaaaacgacggccagtgaattcgagctcggtacccggggatcctctagagtcgacctgcaggcatgcaagcttggcgtaatcatggtcatagctgtttcctgtgtgaaattgttatccgctcacaattccacacaacatacgagccggaagcataaagtgtaaagcctggggtgcctaatgagtgagctaactcacattaattgcgttgcgctcactgcccgctttccagtcgggaaacctgtcgtgccagctgcattaatgaatcggccaacgcgcggggagaggcggtttgcgtattgggcgctcttccgcttcctcgctcactgactcgctgcgctcggtcgttcggctgcggcgagcggtatcagctcactcaaaggcggtaatacggttatccacagaatcaggggataacgcaggaaagaacatgtgagcaaaaggccagcaaaaggccaggaaccgtaaaaaggccgcgttgctggcgtttttccataggctccgcccccctgacgagcatcacaaaaatcgacgctcaagtcagaggtggcgaaacccgacaggactataaagataccaggcgtttccccctggaagctccctcgtgcgctctcctgttccgaccctgccgcttaccggatacctgtccgcctttctcccttcgggaagcgtggcgctttctcaatgctcacgctgtaggtatctcagttcggtgtaggtcgttcgctccaagctgggctgtgtgcacgaaccccccgttcagcccgaccgctgcgccttatccggtaactatcgtcttgagtccaacccggtaagacacgacttatcgccactggcagcagccactggtaacaggattagcagagcgaggtatgtaggcggtgctacagagttcttgaagtggtggcctaactacggctacactagaaggacagtatttggtatctgcgctctgctgaagccagttaccttcggaaaaagagttggtagctcttgatccggcaaacaaaccaccgctggtagcggtggtttttttgtttgcaagcagcagattacgcgcagaaaaaaaggatctcaagaagatcctttgatcttttctacggggtctgacgctcagtggaacgaaaactcacgttaagggattttggtcatgagattatcaaaaaggatcttcacctagatccttttggggtgggcgaagaactccagcatgagatccccgcgctggaggatcatccagccctgatagaaacagaagccactggagcacctcaaaaacaccatcatacactaaatcagtaagttggcagcatcacccgacgcactttgcgccgaataaatacctgtgacggaagatcacttcgcagaataaataaatcctggtgtccctgttgataccgggaagccctgggccaacttttggcgaaaatgagacgttgatcggcacgtaagaggttccaactttcaccataatgaaataagatcactaccgggcgtattttttgagttatcgagattttcaggagctgatagaaacagaagccactggagcacctcaaaaacaccatcatacactaaatcagtaagttggcagcatcacccgacgcactttgcgccgaataaatacctgtgacggaagatcacttcgcagaataaataaatcctggtgtccctgttgataccgggaagccctgggccaacttttggcgaaaatgagacgttgatcggcacgtaagaggttccaactttcaccataatgaaataagatcactaccgggcgtattttttgagttatcgagattttcaggagctctttggcatcgtctctcgcctgtcccctcagttcagtaatttcctgcatttgcctgtttccagtcggtagatattccacaaaacagcagggaagcagcgcttttccgctgcataaccctgcttcggggtcattatagcgattttttcggtatatccatcctttttcgcacgatatacaggattttgccaaagggttcgtgtagactttccttggtgtatccaacggcgtcagccgggcaggataggtgaagtaggcccacccgcgagcgggtgttccttcttcactgtcccttattcgcacctggcggtgctcaacgggaatcctgctctgcgaggctggccggctaccgccggcgtaacagatgagggcaagcggatggctgatgaaaccaagccaaccaggaagggcagcccacctatcaaggtgtactgccttccagacgaacgaagagcgattgaggaaaaggcggcggcggccggcatgagcctgtcggcctacctgctggccgtcggccagggctacaaaatcacgggcgtcgtggactatgagcacgtccgcgagggcgtcccggaaaacgattccgaagcccaacctttcatagaaggcggcggtggaatcgaaatctcgtgatggcaggttgggcgtcgcttggtcggtcatttcgaaaaaggttaggaatacggttagccatttgcctgcttttatatagttcatatgggattcacctttatgttgataagaaataaaagaaaatgccaataggatatcggcattttcttttgcgtttttatttgttaactgttaattgtccttgttcaaggatgctgtctttgacaacagatgttttcttgcctttgatgttcagcaggaagctcggcgcaaacgttgattgtttgtctgcgtagaatcctctgtttgtcatatagcttgtaatcacgacattgtttcctttcgcttgaggtacagcgaagtgtgagtaagtaaaggttacatcgttaggcggatcaagatccatttttaacacaaggccagttttgttcagcggcttgtatgggccagttaaagaattagaaacataaccaagcatgtaaatatcgttagacgtaatgccgtcaatcgtcatttttgatccgcgggagtcagtgaacaggtaccatttgccgttcattttaaagacgttcgcgcgttcaatttcatctgttactgtgttagatgcaatcagcggtttcatcacttttttcagtgtgtaatcatcgtttagctcaatcataccgagagcgccgtttgctaactcagccgtgcgttttttatcgctttgcagaagtttttgactttcttgacggaagaatgatgtgcttttgccatagtatgctttgttaaataaagattcttcgccttggtagccatcttcagttccagtgtttgcttcaaatactaagtatttgtggcctttatcttctacgtagtgaggatctctcagcgtatggttgtcgcctgagctgtagttgccttcatcgatgaactgctgtacattttgatacgtttttccgtcaccgtcaaagattgatttataatcctctacaccgttgatgttcaaagagctgtctgatgctgatacgttaacttgtgcagttgtcagtgtttgtttgccgtaatgtttaccggagaaatcagtgtagaataaacggatttttccgtcagatgtaaatgtggctgaacctgaccattcttgtgtttggtcttttaggatagaatcatttgcatcgaatttgtcgctgtctttaaagacgcggccagcgtttttccagctgtcaatagaagtttcgccgactttttgatagaacatgtaaatcgatgtgtcatccgcatttttaggatctccggctaatgcaaagacgatgtggtagccgtgatagtttgcgacagtgccgtcagcgttttgtaatggccagctgtcccaaacgtccaggccttttgcagaagagatatttttaattgtggacgaatcaaattcagaaacttgatatttttcatttttttgctgttcagggatttgcagcatatcatggcgtgtaatatgggaaatgccgtatgtttccttatatggcttttggttcgtttctttcgcaaacgcttgagttgcgcctcctgccagcagtgcggtagtaaaggttaatactgttgcttgttttgcaaactttttgatgttcatcgttcatgtctccttttttatgtactgtgttagcggtctgcttcttccagccctcctgtttgaagatggcaagttagttacgcacaataaaaaaagacctaaaatatgtaaggggtgacgccaaagtatacactttgccctttacacattttaggtcttgcctgctttatcagtaacaaacccgcgcgatttacttttcgacctcattctattagactctcgtttggattgcaactggtctattttcctcttttgtttgatagaaaatcataaaaggatttgcagactacgggcctaaagaactaaaaaatctatctgtttcttttcattctctgtattttttatagtttctgttgcatgggcataaagttgcctttttaatcacaattcagaaaatatcataatatctcatttcactaaataatagtgaacggcaggtatatgtgatgggttaaaaaggatcaccccagagtcccgctcagaagaactcgtcaagaaggcgatagaaggcgatgcgctgcgaatcgggagcggcgataccgtaaagcacgaggaagcggtcagcccattcgccgccaagctcttcagcaatatcacgggtagccaacgctatgtcctgatagcggtccgccacacccagccggccacagtcgatgaatccagaaaagcggccattttccaccatgatattcggcaagcaggcatcgccatgggtcacgacgagatcctcgccgtcgggcatccgcgccttgagcctggcgaacagttcggctggcgcgagcccctgatgctcttcgtccagatcatcctgatcgacaagaccggcttccatccgagtacgtgctcgctcgatgcgatgtttcgcttggtggtcgaatgggcaggtagccggatcaagcgtatgcagccgccgcattgcatcagccatgatggatactttctcggcaggagcaaggtgagatgacaggagatcctgccccggcacttcgcccaatagcagccagtcccttcccgcttcagtgacaacgtcgagacagctgcgcaaggaacgcccgtcgtggccagccacgatagccgcgctgcctcgtcttggagttcattcagggcaccggacaggtcggtcttgacaaaaagaaccgggcgcccctgcgctgacagccggaacacggcggcatcagagcagccgattgtctgttgtgcccagtcatagccgaatagcctctccacccaagcggccggagaacctgcgtgcaatccatcttgttcaatcatgcgaaacgatcctcatcctgtctcttgatcagatcttgatcccctgcgccatcagatccttggcggcaagaaagccatccagtttactttgcagggcttcccaaccttaccagagggcgccccagctggcaattccg

SEQ ID NO: 12 - DNA, 40 bp, synthetic construct
  misc_feature 1..40: note = Pn*_NCgl0867_F primer
  source 1..40: mol_type = other DNA
tgaattcgagctcggtacccatcgacaaacgcttcaacaa

SEQ ID NO: 13 - DNA, 40 bp, synthetic construct
  misc_feature 1..40: note = Pn*_NCgl0867_R primer
  source 1..40: mol_type = other DNA
gtcgactctagaggatcccccccgtttcaacgcggcgttc

SEQ ID NO: 14 - DNA, 40 bp, synthetic construct
  misc_feature 1..40: note = Pn*_NCgl1062_F primer
  source 1..40: mol_type = other DNA
tgaattcgagctcggtaccccatttcggcgcccatcacca

SEQ ID NO: 15 - DNA, 40 bp, synthetic construct
  misc_feature 1..40: note = Pn*_NCgl1062_R primer
  source 1..40: mol_type = other DNA
gtcgactctagaggatccccaggtggaaggccgcctgagt

SEQ ID NO: 16 - DNA, 40 bp, synthetic construct
  misc_feature 1..40: note = Pn*_NCgl2412_F primer
  source 1..40: mol_type = other DNA
tgaattcgagctcggtacccattctccaccggctcccacc

SEQ ID NO: 17 - DNA, 40 bp, synthetic construct
  misc_feature 1..40: note = Pn*_NCgl2412_R primer
  source 1..40: mol_type = other DNA
gtcgactctagaggatccccgagctgaacgaagctatctt

SEQ ID NO: 18 - DNA, 40 bp, synthetic construct
  misc_feature 1..40: note = Pn*_NCgl1224_F primer
  source 1..40: mol_type = other DNA
tgaattcgagctcggtacccatccccgtgctcaaagtcgt

SEQ ID NO: 19 - DNA, 40 bp, synthetic construct
  misc_feature 1..40: note = Pn*_NCgl1224_R primer
  source 1..40: mol_type = other DNA
gtcgactctagaggatcccccagcggtggtcttgacctcg

SEQ ID NO: 20 - DNA, 40 bp, synthetic construct
  misc_feature 1..40: note = Pn*_NCgl2581_F primer
  source 1..40: mol_type = other DNA
tgaattcgagctcggtacccgttgggtgctcttatctgca

SEQ ID NO: 21 - DNA, 40 bp, synthetic construct
  misc_feature 1..40: note = Pn*_NCgl2581_R primer
  source 1..40: mol_type = other DNA
gtcgactctagaggatccccgataccaatgaacaccggat

SEQ ID NO: 22 - DNA, 40 bp, synthetic construct
  misc_feature 1..40: note = Pn*_NCgl2658_F primer
  source 1..40: mol_type = other DNA
tgaattcgagctcggtacccatgcgtctcagccactggga

SEQ ID NO: 23 - DNA, 40 bp, synthetic construct
  misc_feature 1..40: note = Pn*_NCgl2658_R primer
  source 1..40: mol_type = other DNA
gtcgactctagaggatccccagattcctgctggacctgca

SEQ ID NO: 24 - DNA, 41 bp, synthetic construct
  misc_feature 1..41: note = Pn*_NCgl2046_F primer
  source 1..41: mol_type = other DNA
tgaattcgagctcggtacccttcatcgtcatcatcgctggt

SEQ ID NO: 25 - DNA, 40 bp, synthetic construct
  misc_feature 1..40: note = Pn*_NCgl2046_R primer
  source 1..40: mol_type = other DNA
gtcgactctagaggatccccgtaggaacgaacatcctgca

SEQ ID NO: 26 - DNA, 35 bp, synthetic construct
  misc_feature 1..35: note = Pn*_NCgl0780_F primer
  source 1..35: mol_type = other DNA
tgaattcgagctcggtacccctgtttcgagatgag

SEQ ID NO: 27 - DNA, 35 bp, synthetic construct
  misc_feature 1..35: note = Pn*_NCgl0780_R primer
  source 1..35: mol_type = other DNA
gtcgactctagaggatcccccccgccaacgcaata

SEQ ID NO: 28 - DNA, 35 bp, synthetic construct
  misc_feature 1..35: note = Pn*_NCgl1896_F primer
  source 1..35: mol_type = other DNA
tgaattcgagctcggtacccctgaccgaccaggaa

SEQ ID NO: 29 - DNA, 35 bp, synthetic construct
  misc_feature 1..35: note = Pn*_NCgl1896_R primer
  source 1..35: mol_type = other DNA
gtcgactctagaggatccccggatgagtctcggtt

SEQ ID NO: 30 - DNA, 35 bp, synthetic construct
  misc_feature 1..35: note = Pn*_NCgl2356_F primer
  source 1..35: mol_type = other DNA
tgaattcgagctcggtacccccactgccatggctg

SEQ ID NO: 31 - DNA, 35 bp, synthetic construct
  misc_feature 1..35: note = Pn*_NCgl2356_R primer
  source 1..35: mol_type = other DNA
gtcgactctagaggatccccgttgaggcgggcgag

SEQ ID NO: 32 - DNA, 18 bp, synthetic construct
  misc_feature 1..18: note = pNCgl0867_F primer
  source 1..18: mol_type = other DNA
aatcaatcttcgcactcg

SEQ ID NO: 33 - DNA, 18 bp, synthetic construct
  misc_feature 1..18: note = pNCgl0867_R primer
  source 1..18: mol_type = other DNA
tctcttgctcgatgaacg

SEQ ID NO: 34 - DNA, 18 bp, synthetic construct
  misc_feature 1..18: note = pNCgl1062_F primer
  source 1..18: mol_type = other DNA
actcgaattcaccgaaac

SEQ ID NO: 35 - DNA, 18 bp, synthetic construct
  misc_feature 1..18: note = pNCgl1062_R primer
  source 1..18: mol_type = other DNA
ctcatccacgtctactgt

SEQ ID NO: 36 - DNA, 18 bp, synthetic construct
  misc_feature 1..18: note = pNCgl2412_F primer
  source 1..18: mol_type = other DNA
ctacggacacatggaata

SEQ ID NO: 37 - DNA, 18 bp, synthetic construct
  misc_feature 1..18: note = pNCgl2412_R primer
  source 1..18: mol_type = other DNA
tcttccacatccatcgtc

SEQ ID NO: 38 - DNA, 18 bp, synthetic construct
  misc_feature 1..18: note = pNCgl1224_F primer
  source 1..18: mol_type = other DNA
taaagaccgaaacactcg

SEQ ID NO: 39 - DNA, 18 bp, synthetic construct
  misc_feature 1..18: note = pNCgl1224_R primer
  source 1..18: mol_type = other DNA
cgttggtgaagatttctg

SEQ ID NO: 40 - DNA, 18 bp, synthetic construct
  misc_feature 1..18: note = pNCgl2581_F primer
  source 1..18: mol_type = other DNA
cttatcgacgtctccctt

SEQ ID NO: 41 - DNA, 18 bp, synthetic construct
  misc_feature 1..18: note = pNCgl2581_R primer
  source 1..18: mol_type = other DNA
tgggagcgagttcttgga

SEQ ID NO: 42 - DNA, 17 bp, synthetic construct
  misc_feature 1..17: note = pNCgl2658_F primer
  source 1..17: mol_type = other DNA
attgatgacacttcagg

SEQ ID NO: 43 - DNA, 18 bp, synthetic construct
  misc_feature 1..18: note = pNCgl2658_R primer
  source 1..18: mol_type = other DNA
caacaccataacggatca

SEQ ID NO: 44 - DNA, 19 bp, synthetic construct
  misc_feature 1..19: note = pNCgl2046_F primer
  source 1..19: mol_type = other DNA
acgcagagtctgcttgaac

SEQ ID NO: 45 - DNA, 17 bp, synthetic construct
  misc_feature 1..17: note = pNCgl2046_R primer
  source 1..17: mol_type = other DNA
acaggaacatagatgcg

SEQ ID NO: 46 - DNA, 20 bp, synthetic construct
  misc_feature 1..20: note = pNCgl0780_F primer
  source 1..20: mol_type = other DNA
gtccctagtacgagaggacc

SEQ ID NO: 47 - DNA, 20 bp, synthetic construct
  misc_feature 1..20: note = pNCgl0780_R primer
  source 1..20: mol_type = other DNA
ttatgcggcgaattaacgat

SEQ ID NO: 48 - DNA, 20 bp, synthetic construct
  misc_feature 1..20: note = pNCgl1896_F primer
  source 1..20: mol_type = other DNA
caagtcccgtttctttgatc

SEQ ID NO: 49 - DNA, 20 bp, synthetic construct
  misc_feature 1..20: note = pNCgl1896_R primer
  source 1..20: mol_type = other DNA
ccgccatttttccttctctc

SEQ ID NO: 50 - DNA, 20 bp, synthetic construct
  misc_feature 1..20: note = pNCgl2356_F primer
  source 1..20: mol_type = other DNA
tagctcgacttggcgctgaa

SEQ ID NO: 51 - DNA, 20 bp, synthetic construct
  misc_feature 1..20: note = pNCgl2356_R primer
  source 1..20: mol_type = other DNA
gtttttattggcggtggtga

SEQ ID NO: 52 - DNA, 396 bp, synthetic construct
  misc_feature 1..396: note = Pn_NCgl0867
  source 1..396: mol_type = other DNA
gacgtcaaaaagttttagcactataacgttatgacgttttagtgctaaagtgtggcttgtcagattcgtgttggtcgtgcgcccgtatggtgatttgagacagggtttaggagaattagttccatgtcgaatcgcacgtcatcttcaccgaagaattcaaagcaggagctgtgcaactcgtcgtatcctcagggcgctcggtcaaggaagtggccaccgagttgggtatcaaagaaggaacactgagcgcgtgggtaagaacctggagggccgagcatccagacgccggtgtggatgaaccaggcccagtcgaatgggcgaaatacaaggccctgcaggctgagaacgccgcgttgaaacgggaaaacgagttttggggaaaagccagcgccttct

SEQ ID NO: 53 - DNA, 164 bp, synthetic construct
  misc_feature 1..164: note = Pn_NCgl1062
  source 1..164: mol_type = other DNA
cccccatttggttcgcagccgatgaggagttacgcactatcgactccatcgaaggccaagcaaattggtcaatcaagcgtgaatccggcttccatgagccagttgcccgcctcaaagcttgacccattttcataaccagtgccatgtgggtttacggttgatac

SEQ ID NO: 54 - DNA, 164 bp, synthetic construct
  misc_feature 1..164: note = Pn_NCgl2412
  source 1..164: mol_type = other DNA
ctaggacactggaacctaaatccagcgcgtctgccaattccgccacaagcgcttaatgcgggttttactatacatggtgtagtcccaaattaactaatgcgggtgaccaactgcaccgtaaaaaaaattcgcttatcgtaaatcagcaggtagaataacactct

SEQ ID NO: 55 - DNA, 180 bp, synthetic construct
  misc_feature 1..180: note = Pn_NCgl1124
  source 1..180: mol_type = other DNA
acagcaattaatctgattgcacctgctgcataaatgtgactagtcaaacaccgtctaattacatgtgtgtggtagaacaataatgtagttgtctgcccaagcgagttaaactcccacgatttacagtggggggcagacatcttttcaccaaaatttttacgaaaggcgagattttctccc

SEQ ID NO: 56 - DNA, 232 bp, synthetic construct
  misc_feature 1..232: note = Pn_NCgl2581
  source 1..232: mol_type = other DNA
aaatttgtgggaaccgaccgacaagtccgtggcctaatcatggacgtactgcgcaatgccaccgcacctgtgccactatccgcgattgatgtcgtgtggcctgacgatgcccaacgctcccgggcgctgttttcgctcattgaggacggactcgcggaacaaaatgaggcgggttatttccacctgccacggtaaaccactgcgcgcctgcaaaaaacagtaggtttaagta

SEQ ID NO: 57 - DNA, 326 bp, synthetic construct
  misc_feature 1..326: note = Pn_NCgl2658
  source 1..326: mol_type = other DNA
agcacaaatgcttattgccgtagaaaacaatacggagcggttacaagttgcgaagcaccctttgcaaagtttttagcggtactttacagctcttcaccccccattaatggggtctatgaaagcgcgcagcgtgacaaatctgaccccagcaaagcccccaatactccccgactggcctttattagtctgcacttaccacgtatcatggagggttgatagcagggcaccattagcagtcgcaccccgataggagtcgaatctacaagtggaacccccgctcacatactccacattttttagaacccctttaaggaatcgaactttat

SEQ ID NO: 58 - DNA, 235 bp, synthetic construct
  misc_feature 1..235: note = Pn_NCgl2046
  source 1..235: mol_type = other DNA
agtacttcgacgcaaagacaaaacttttctcctggcaataaatatgcggatttactatggaaacaagatagaagattggatagcgaaagctatcctcaactcgtggaaagtgtagtgccacaaccacagtattggctagaaaacaatctatagcattgttctacaaagagcttgttggaaataaaacctatgccaaagtaggtgcaattctaggagaagattacactagtcaacc

SEQ ID NO: 59 - DNA, 183 bp, synthetic construct
  misc_feature 1..183: note = Pn_NCgl0780
  source 1..183: mol_type = other DNA
ggggtgtggtggatacacatggttgtgtgttcaccgcaccctctctttttttgtgtttgtgggggtcttgggccccttgtgcacgcggcacgcacgctgggggcaagcgtcgacaagcacaaactttttgcttaattgaatcctttgcgcaccaatcaatgggggatcaaatatagtagctgc

SEQ ID NO: 60 - DNA, 200 bp, synthetic construct
  misc_feature 1..200: note = Pn_NCgl1896
  source 1..200: mol_type = other DNA
cgcaaagctcacacccacgagctaaaaattcatatagttaagacaacatttttggctgtaaaagacagccgtaaaaacctcttgctcgtgtcaattgttcttatcggaatgtggcttgggcgattgttatgcaaaagttgttaggttttttgcggggttgtttaacccccaaatgagggaagaaggtaaccttgaactct

SEQ ID NO: 61 - DNA, 283 bp, synthetic construct
  misc_feature 1..283: note = Pn_NCgl2356
  source 1..283: mol_type = other DNA
gttttctagataacaaggccagcacagaccaccatatctacgaccccaaaaaccgactccaagctccgcggcgacgaagccgcgctcgcgccaccgaccaagcagccggtccaggtttaaagattttgcttttcgacgctcccctccacctcattcaatgcggcggaggggatttccttgcatgttaagcctataggaaaaagtgtttgcatatcacccttgtattcgaacacgtgagcgggtagagtgggtggtaacaacacggggaaagggggaagacacc